European Patent Specification EP 4 200 591 B1, published November 20, 2024. Title: BIOSENSOR USING PARTICLE MOTION. Applicant: Technische Universiteit Eindhoven. The sequence listing filed with the application follows.

SEQUENCE LISTING (4 sequences)

SEQ ID NO: 1 - DNA, 11 bp, Artificial Sequence
  Particle binder
agcatggcact

SEQ ID NO: 2 - DNA, 22 bp, Artificial Sequence
  Analyte
tcgtaccgtgagtaataatgcg

SEQ ID NO: 3 - DNA, 31 bp, Artificial Sequence
  Detecting
cattattacaagctaagctcttgcactgacg

SEQ ID NO: 4 - DNA, 25 bp, Artificial Sequence
  Surface binder
cgattccagaacgtgactgcttttt